European Patent Application EP 4 293 115 A1, published December 20, 2023. Title: 具有启动子活性的多核苷酸及其在生产目标化合物中的用途. Applicant: 中国科学院天津工业生物技术研究所. The sequence listing filed with the application follows.

SEQUENCE LISTING (70 sequences)

SEQ ID NO: 1 - DNA, 243 bp, Artificial Sequence
  sequence of 243 bp PNCgl1418
taaaactcgcgatgaagtagaaaaacaacgcaacacttaagacacctgtgagtttcaaactccccattatcgccttagtcaggcggtagtggggagtttttgtttatgcaggtggcgcgattcttagatttcataagggtaacagatctgtttctatgtattaaagatcacaccgagtggtggaatttcctcaagtgatttacccacaatggactttgttgatacccaattcgagaaaggcca

SEQ ID NO: 2 - DNA, 203 bp, Artificial Sequence
  sequence of 203 bp PNCgl1418
gacacctgtgagtttcaaactccccattatcgccttagtcaggcggtagtggggagtttttgtttatgcaggtggcgcgattcttagatttcataagggtaacagatctgtttctatgtattaaagatcacaccgagtggtggaatttcctcaagtgatttacccacaatggactttgttgatacccaattcgagaaaggcca

SEQ ID NO: 3 - DNA, 145 bp, Artificial Sequence
  sequence of 145 bp PNCgl1418
tttgtttatgcaggtggcgcgattcttagatttcataagggtaacagatctgtttctatgtattaaagatcacaccgagtggtggaatttcctcaagtgatttacccacaatggactttgttgatacccaattcgagaaaggcca

SEQ ID NO: 4 - DNA, 94 bp, Artificial Sequence
  sequence of 94 bp PNCgl1418
gtttctatgtattaaagatcacaccgagtggtggaatttcctcaagtgatttacccacaatggactttgttgatacccaattcgagaaaggcca

SEQ ID NO: 5 - DNA, 349 bp, Artificial Sequence
  sequence of Ptuf
agatcgtttagatccgaaggaaaacgtcgaaaagcaatttgcttttcgacgccccaccccgcgcgttttagcgtgtcagtaggcgcgtagggtaagtggggtagcggcttgttagatatcttgaaatcggctttcaacagcattgatttcgatgtatttagctggccgttaccctgcgaatgtccacagggtagctggtagtttgaaaatcaacgccgttgcccttaggattcagtaactggcacattttgtaatgcgctagatctgtgtgctcagtcttccaggctgcttatcacagtgaaagcaaaaccaattcgtggctgcgaaagtcgtagccaccacgaagtcc

SEQ ID NO: 6 - DNA, 40 bp, Artificial Sequence
  primer sequence
cttttcaccagtgagacgggtaaaactcgcgatgaagtag

SEQ ID NO: 7 - DNA, 41 bp, Artificial Sequence
  primer sequence
gttcttctcctttactcatcattggcctttctcgaattggg

SEQ ID NO: 8 - DNA, 26 bp, Artificial Sequence
  primer sequence
atgagtaaaggagaagaacttttcac

SEQ ID NO: 9 - DNA, 20 bp, Artificial Sequence
  primer sequence
cccgtctcactggtgaaaag

SEQ ID NO: 10 - DNA, 39 bp, Artificial Sequence
  primer sequence
caccagtgagacgggagatcgtttagatccgaaggaaaa

SEQ ID NO: 11 - DNA, 38 bp, Artificial Sequence
  primer sequence
ctcgaattgggtatcaacggacttcgtggtggctacga

SEQ ID NO: 12 - DNA, 23 bp, Artificial Sequence
  primer sequence
gttgatacccaattcgagaaagg

SEQ ID NO: 13 - DNA, 20 bp, Artificial Sequence
  primer sequence
cccgtctcactggtgaaaag

SEQ ID NO: 14 - DNA, 23 bp, Artificial Sequence
  primer sequence
gacacctgtgagtttcaaactcc

SEQ ID NO: 15 - DNA, 20 bp, Artificial Sequence
  primer sequence
cccgtctcactggtgaaaag

SEQ ID NO: 16 - DNA, 19 bp, Artificial Sequence
  primer sequence
tttgtttatgcaggtggcg

SEQ ID NO: 17 - DNA, 20 bp, Artificial Sequence
  primer sequence
cccgtctcactggtgaaaag

SEQ ID NO: 18 - DNA, 26 bp, Artificial Sequence
  primer sequence
gtttctatgtattaaagatcacaccg

SEQ ID NO: 19 - DNA, 20 bp, Artificial Sequence
  primer sequence
cccgtctcactggtgaaaag

SEQ ID NO: 20 - DNA, 40 bp, Artificial Sequence; identical to SEQ ID NO: 6
  primer sequence

SEQ ID NO: 21 - DNA, 40 bp, Artificial Sequence
  primer sequence
ttcttgataaattgacaccattggcctttctcgaattggg

SEQ ID NO: 22 - DNA, 30 bp, Artificial Sequence
  primer sequence
gtgtcaatttatcaagaatttgttaataaa

SEQ ID NO: 23 - DNA, 26 bp, Artificial Sequence
  primer sequence
gcggatacatatttgaatgtatttag

SEQ ID NO: 24 - DNA, 46 bp, Artificial Sequence
  primer sequence
acacgcgtctgagcagtattcatgagacaataaccctgataaatgc

SEQ ID NO: 25 - DNA, 20 bp, Artificial Sequence
  primer sequence
cccgtctcactggtgaaaag

SEQ ID NO: 26 - DNA, 40 bp, Artificial Sequence
  primer sequence
cattcaaatatgtatccgcgagagtcaattcagggtggtg

SEQ ID NO: 27 - DNA, 21 bp, Artificial Sequence
  primer sequence
aatactgctcagacgcgtgtc

SEQ ID NO: 28 - DNA, 30 bp, Artificial Sequence; identical to SEQ ID NO: 22
  primer sequence

SEQ ID NO: 29 - DNA, 20 bp, Artificial Sequence
  primer sequence
cccgtctcactggtgaaaag

SEQ ID NO: 30 - DNA, 39 bp, Artificial Sequence
  primer sequence
agcggcatgcatttacgtttaaaactcgcgatgaagtag

SEQ ID NO: 31 - DNA, 41 bp, Artificial Sequence
  primer sequence
agatttccatgatcaccatcattggcctttctcgaattggg

SEQ ID NO: 32 - DNA, 26 bp, Artificial Sequence
  primer sequence
atggtgatcatggaaatcttcattac

SEQ ID NO: 33 - DNA, 44 bp, Artificial Sequence
  primer sequence
gtctgtttcctgtgtgaaactaacccatcaacatcagtttgatg

SEQ ID NO: 34 - DNA, 23 bp, Artificial Sequence
  primer sequence
tttcacacaggaaacagaccatg

SEQ ID NO: 35 - DNA, 21 bp, Artificial Sequence
  primer sequence
aacgtaaatgcatgccgcttc

SEQ ID NO: 36 - DNA, 60 bp, Corynebacterium glutamicum
tattaaagatcacaccgagtggtggaatttcctcaagtgatttacccacaatggactttg

SEQ ID NO: 37 - DNA, 243 bp, Artificial Sequence
  sequence of 35P1
taaaactcgcgatgaagtagaaaaacaacgcaacacttaagacacctgtgagtttcaaactccccattatcgccttagtcaggcggtagtggggagtttttgtttatgcaggtggcgcgattcttagatttcataagggtaacagatctgtttctatgtattaaagatctacttgcagagtggaatttcctcaagtgatttacccacaatggactttgttgatacccaattcgagaaaggcca

SEQ ID NO: 38 - DNA, 243 bp, Artificial Sequence
  sequence of 35P2
taaaactcgcgatgaagtagaaaaacaacgcaacacttaagacacctgtgagtttcaaactccccattatcgccttagtcaggcggtagtggggagtttttgtttatgcaggtggcgcgattcttagatttcataagggtaacagatctgtttctatgtattaaagatcagtgctgaaagtggaatttcctcaagtgatttacccacaatggactttgttgatacccaattcgagaaaggcca

SEQ ID NO: 39 - DNA, 243 bp, Artificial Sequence
  sequence of 35P3
taaaactcgcgatgaagtagaaaaacaacgcaacacttaagacacctgtgagtttcaaactccccattatcgccttagtcaggcggtagtggggagtttttgtttatgcaggtggcgcgattcttagatttcataagggtaacagatctgtttctatgtattaaagatcgcacgaaagggtggaatttcctcaagtgatttacccacaatggactttgttgatacccaattcgagaaaggcca

SEQ ID NO: 40 - DNA, 243 bp, Artificial Sequence
  sequence of 35P4
taaaactcgcgatgaagtagaaaaacaacgcaacacttaagacacctgtgagtttcaaactccccattatcgccttagtcaggcggtagtggggagtttttgtttatgcaggtggcgcgattcttagatttcataagggtaacagatctgtttctatgtattaaagatctatctagagggtggaatttcctcaagtgatttacccacaatggactttgttgatacccaattcgagaaaggcca

SEQ ID NO: 41 - DNA, 243 bp, Artificial Sequence
  sequence of 35P5
taaaactcgcgatgaagtagaaaaacaacgcaacacttaagacacctgtgagtttcaaactccccattatcgccttagtcaggcggtagtggggagtttttgtttatgcaggtggcgcgattcttagatttcataagggtaacagatctgtttctatgtattaaagatcaggcttgtcggtggaatttcctcaagtgatttacccacaatggactttgttgatacccaattcgagaaaggcca

SEQ ID NO: 42 - DNA, 243 bp, Artificial Sequence
  sequence of 35P6
taaaactcgcgatgaagtagaaaaacaacgcaacacttaagacacctgtgagtttcaaactccccattatcgccttagtcaggcggtagtggggagtttttgtttatgcaggtggcgcgattcttagatttcataagggtaacagatctgtttctatgtattaaagatccgcttctttcgtggaatttcctcaagtgatttacccacaatggactttgttgatacccaattcgagaaaggcca

SEQ ID NO: 43 - DNA, 243 bp, Artificial Sequence
  sequence of 35P7
taaaactcgcgatgaagtagaaaaacaacgcaacacttaagacacctgtgagtttcaaactccccattatcgccttagtcaggcggtagtggggagtttttgtttatgcaggtggcgcgattcttagatttcataagggtaacagatctgtttctatgtattaaagatctaactcttgggtggaatttcctcaagtgatttacccacaatggactttgttgatacccaattcgagaaaggcca

SEQ ID NO: 44 - DNA, 243 bp, Artificial Sequence
  sequence of 35P8
taaaactcgcgatgaagtagaaaaacaacgcaacacttaagacacctgtgagtttcaaactccccattatcgccttagtcaggcggtagtggggagtttttgtttatgcaggtggcgcgattcttagatttcataagggtaacagatctgtttctatgtattaaagatcccaagttccagtggaatttcctcaagtgatttacccacaatggactttgttgatacccaattcgagaaaggcca

SEQ ID NO: 45 - DNA, 243 bp, Artificial Sequence
  sequence of 35P9
taaaactcgcgatgaagtagaaaaacaacgcaacacttaagacacctgtgagtttcaaactccccattatcgccttagtcaggcggtagtggggagtttttgtttatgcaggtggcgcgattcttagatttcataagggtaacagatctgtttctatgtattaaagatccggtgccacagtggaatttcctcaagtgatttacccacaatggactttgttgatacccaattcgagaaaggcca

SEQ ID NO: 46 - DNA, 243 bp, Artificial Sequence
  sequence of 35P10
taaaactcgcgatgaagtagaaaaacaacgcaacacttaagacacctgtgagtttcaaactccccattatcgccttagtcaggcggtagtggggagtttttgtttatgcaggtggcgcgattcttagatttcataagggtaacagatctgtttctatgtattaaagatcagcagttagggtggaatttcctcaagtgatttacccacaatggactttgttgatacccaattcgagaaaggcca

SEQ ID NO: 47 - DNA, 243 bp, Artificial Sequence
  sequence of 35P11
taaaactcgcgatgaagtagaaaaacaacgcaacacttaagacacctgtgagtttcaaactccccattatcgccttagtcaggcggtagtggggagtttttgtttatgcaggtggcgcgattcttagatttcataagggtaacagatctgtttctatgtattaaagatcagataaataagtggaatttcctcaagtgatttacccacaatggactttgttgatacccaattcgagaaaggcca

SEQ ID NO: 48 - DNA, 243 bp, Artificial Sequence
  sequence of 35P12
taaaactcgcgatgaagtagaaaaacaacgcaacacttaagacacctgtgagtttcaaactccccattatcgccttagtcaggcggtagtggggagtttttgtttatgcaggtggcgcgattcttagatttcataagggtaacagatctgtttctatgtattaaagatcatcgatctaggtggaatttcctcaagtgatttacccacaatggactttgttgatacccaattcgagaaaggcca

SEQ ID NO: 49 - DNA, 35 bp, Artificial Sequence
  sequence of primer 1418mutant-F
  misc_feature (1)..(10): n is a, c, g, or t
nnnnnnnnnngtggaatttcctcaagtgatttacc

SEQ ID NO: 50 - DNA, 33 bp, Artificial Sequence
  sequence of primer 1418mutant-R
gatctttaatacatagaaacagatctgttaccc

SEQ ID NO: 51 - DNA, 34 bp, Artificial Sequence
  sequence of primer 35P7-F
taactcttgggtggaatttcctcaagtgatttac

SEQ ID NO: 52 - DNA, 51 bp, Artificial Sequence
  sequence of primer 35P7-R1
aaattccacccaagagttagatctttaatacatagaaacagatctgttacc

SEQ ID NO: 53 - DNA, 32 bp, Artificial Sequence
  sequence of primer 35P7-R2
gatctttaatacatagaaacagatctgttacc

SEQ ID NO: 54 - DNA, 22 bp, Artificial Sequence
  sequence of primer pXM-F
caaaggcggtaatacggttatc

SEQ ID NO: 55 - DNA, 21 bp, Artificial Sequence
  sequence of primer pXM-R
aaccgtattaccgcctttgag

SEQ ID NO: 56 - DNA, 384 bp, Corynebacterium glutamicum
gcaccgaaaacagtaactttcccaagaaaaatataagaaaacttccccacacaggccgtgaagagcctgaatttattgatttttcagacagatctggaaatgtgaccaatttgtaacccacccccgctcacctgcatgagtgtggggtctttttgcattcttccagctcccagacttgaaaacgatctgacttttcaccccgaaccttactaaggtcgattcatgttgaaaagagaggtggtgttttcacttcccttttataggcaaagctttaaggagtcttacaggaagaagttaacaccgcccaggggtgcgttggatgatgatcatctacaaacaaacattccgttatgcactcataagatatgacgagaggttttactc

SEQ ID NO: 57 - DNA, 381 bp, Artificial Sequence
  sequence of PproP-1
gcaccgaaaacagtaactttcccaagaaaaatataagaaaacttccccacacaggccgtgaagagcctgaatttattgatttttcagacagatctggaaatgtgaccaatttgtaacccacccccgctcacctgcatgagtgtggggtctttttgcattcttccagctcccagacttgaaaacgatctgacttttcaccccgaaccttactaaggtcgattcatgttgaaaagagaggtggtgttttcacttcccttttataggcaaagctttaaggagtcttacaggaagaagttaacaccgcccaggggtgcgttggatgatgatcatctacaaacaaacattccgttatgcacttgatacccaattcgagaaaggcca

SEQ ID NO: 58 - DNA, 250 bp, Artificial Sequence
  sequence of PproP-2
gcaccgaaaacagtaactttcccaagaaaaatataagaaaacttccccacacaggccgtgaagagcctgaatttattgatttttcagacagatctggaaatgtgaccaatttgtaacccacccccgctcacctgcatgagtgtggggtctttttgcattcttccatattaaagatcacaccgagtggtggaatttcctcaagtgatttacccacaatggactttgttgatacccaattcgagaaaggcca

SEQ ID NO: 59 - DNA, 40 bp, Artificial Sequence
  primer sequence
tttcaccagtgagacggggcaccgaaaacagtaactttcc

SEQ ID NO: 60 - DNA, 47 bp, Artificial Sequence
  primer sequence
ttcttctcctttactcatgagtaaaacctctcgtcatatcttatgag

SEQ ID NO: 61 - DNA, 41 bp, Artificial Sequence
  primer sequence
cgagaaaggccaatgatgagtaaaggagaagaacttttcac

SEQ ID NO: 62 - DNA, 36 bp, Artificial Sequence
  primer sequence
aattgggtatcaagtgcataacggaatgtttgtttg

SEQ ID NO: 63 - DNA, 67 bp, Artificial Sequence
  primer sequence
acaatggactttgttgatacccaattcgagaaaggccaatgatgagtaaaggagaagaacttttcac

SEQ ID NO: 64 - DNA, 68 bp, Artificial Sequence
  primer sequence
gggtaaatcacttgaggaaattccaccactcggtgtgatctttaatatggaagaatgcaaaaagaccc

SEQ ID NO: 65 - DNA, 41 bp, Artificial Sequence
  primer sequence
ttttcaccagtgagacggggcaccgaaaacagtaactttcc

SEQ ID NO: 66 - DNA, 49 bp, Artificial Sequence
  primer sequence
aattcttgataaattgacacgagtaaaacctctcgtcatatcttatgag

SEQ ID NO: 67 - DNA, 40 bp, Artificial Sequence
  primer sequence
attcttgataaattgacaccattggcctttctcgaattgg

SEQ ID NO: 68 - DNA, 40 bp, Artificial Sequence
  primer sequence
gcggcatgcatttacgttgcaccgaaaacagtaactttcc

SEQ ID NO: 69 - DNA, 49 bp, Artificial Sequence
  primer sequence
aagatttccatgatcaccatgagtaaaacctctcgtcatatcttatgag

SEQ ID NO: 70 - DNA, 40 bp, Artificial Sequence
  primer sequence
agatttccatgatcaccatcattggcctttctcgaattgg